European Patent Application EP 4 610 657 A1, published September 3, 2025. Title: MMP12を指標とした免疫介在性炎症性疾患の診断、及びMMP12阻害による免疫介在性炎症性疾患の治療用医薬. Applicant: 慶應義塾. The sequence listing filed with the application follows.

SEQUENCE LISTING (32 sequences)

SEQ ID NO: 1 - protein, 13 aa, synthetic construct
ASVATELRCQCLQ

SEQ ID NO: 2 - protein, 13 aa, synthetic construct
APLATELRCQCLQ

SEQ ID NO: 3 - protein, 13 aa, synthetic construct
ASVVTELRCQCLQ

SEQ ID NO: 4 - protein, 13 aa, synthetic construct
AAVLRELRCVCLQ

SEQ ID NO: 5 - protein, 13 aa, synthetic construct
PRSAKELRCQCIK

SEQ ID NO: 6 - protein, 13 aa, synthetic construct
APIANELRCQCLQ

SEQ ID NO: 7 - protein, 13 aa, synthetic construct
AVVASELRCQCLK

SEQ ID NO: 8 - protein, 13 aa, synthetic construct
AVVASELRCQCLN

SEQ ID NO: 9 - protein, 13 aa, synthetic construct
VIAATELRCVCLT

SEQ ID NO: 10 - protein, 12 aa, synthetic construct
TKTESSSRGPYH

SEQ ID NO: 11 - protein, 14 aa, synthetic construct
DKWVQDYIKDMKEN

SEQ ID NO: 12 - protein, 12 aa, synthetic construct
STNLQKRLRRKD

SEQ ID NO: 13 - protein, 12 aa, synthetic construct
SLSFSTNLQKRL

SEQ ID NO: 14 - protein, 12 aa, synthetic construct
SRNLQERLRRKE

SEQ ID NO: 15 - protein, 12 aa, synthetic construct
SFSSSRNLQERL

SEQ ID NO: 16 - protein, 12 aa, synthetic construct
STNLQESLRRKE

SEQ ID NO: 17 - protein, 12 aa, synthetic construct
SFSLSTNLQESL

SEQ ID NO: 18 - protein, 12 aa, synthetic construct
SINLQKRLKSKE

SEQ ID NO: 19 - protein, 12 aa, synthetic construct
SFSLSINLQKRL

SEQ ID NO: 20 - protein, 14 aa, synthetic construct
LNVQRKAIHELIQV

SEQ ID NO: 21 - protein, 14 aa, synthetic construct
RKAIHELIQVMAEL

SEQ ID NO: 22 - protein, 15 aa, synthetic construct
KRKRSQMLFRGRRAS

SEQ ID NO: 23 - protein, 13 aa, synthetic construct
QVQRQAFNEKIRV

SEQ ID NO: 24 - protein, 14 aa, synthetic construct
RQAFNEKIRVVHQL

SEQ ID NO: 25 - protein, 12 aa, synthetic construct
PESSLRKRKRSR

SEQ ID NO: 26 - protein, 14 aa, synthetic construct
APIANELRSQSLQT

SEQ ID NO: 27 - protein, 13 aa, synthetic construct
AKRNALAVERTAS

SEQ ID NO: 28 - protein, 14 aa, synthetic construct
APRIKKIVQKKLAG

SEQ ID NO: 29 - protein, 14 aa, synthetic construct
ASVVTELRSQSLQT

SEQ ID NO: 30 - protein, 12 aa, synthetic construct
LPRSAKELRSQS

SEQ ID NO: 31 - protein, 13 aa, synthetic construct
PAAAVLRELRSVS

SEQ ID NO: 32 - protein, 14 aa, synthetic construct
ELRSTSLRVTLRVN